European Patent Specification EP 3 677 674 B1, published October 4, 2023. Title: Transaminase mutant and use thereof. Applicant: ASYMCHEM LIFE SCIENCETIANJINCO.,LTD. The sequence listing filed with the application follows.

SEQUENCE LISTING (60 sequences)

SEQ ID NO: 1 - protein, 341 aa, (Actinobacteria sp.) [sequence omitted]

SEQ ID NO: 2 - protein, 341 aa, (Actinobacteria sp.)
MTISKDIDYSTSNLVSVAPGAIREPTPAGSVIQYSDYELDESSPFAGGAAWIEGEYVPAAEARISLFDTGFGHSDATYTVAHVWHGNIFRLKDHIDRVFDGAQKLRLQSPLTKAEVEDITKRCVSLSQLAESFVNITITRGYGARKGEKDLSKLTSQIYIYAIPYLWAFPPEEQIFGTSAIVPRHVRRAGRNTVDPTVKNYQWGDLTAASFEAKDRGARTAILLDADNCVAEGPGFNVVMVKDGKLSSPSRNALPGITRLTVMEMADEMGIEFTLRDITSRELYEADELIACTTGGGITPITSLDGEPLGDGTPGPVTVAIRDRFWAMMDEPSSLVEAIEY

SEQ ID NO: 3 - protein, 341 aa, (Actinobacteria sp.)
MTISKDIDYSTSNLVSVAPGAIREPTPAGSVIQYSDYELDESSPFAGGAAWIEGEYVPAAEARISLFDTGFGHSDLTYTVAHVWHGNIFRLKDHIDRVFDGAQKLRIQSPLTKAEVEDITKRCVSLSQLRESFVNITITRGYGARKGEKDLSKLTSQIYIYAIPYLWAFPPEEQIFGTSAIVPRHVRRAGRNTVDPTVKNYQWGDLTAASFEAKDRGARTAILLDADNCVAEGPGFNVVMVKDGKLSSPSRNALPGITRLTVMEMADEMGIEFTLRDITSRELYEADELIAVTTGGGITPITSLDGEPLGDGTPGPVTVAIRDRFWAMMDEPSSLVEAIEY

SEQ ID NO: 4 - protein, 341 aa, (Actinobacteria sp.)
MTISKDIDYSTSNLVSVAPGAIREPTPAGSVIQYSDYELDESNPFAGGAAWIEGEYVPAAEARISLFDTGFLHSDLTYTVAHVWHGNIFRLKDHIDRVFDGAQKLRLQSPLTKAEVEDITKRCVSLSQLRESFVNITITRGYGARKGEKDLSKLTSQIYIYAIPYLWAFPPEEQIFGTSAIVPRHVRRAGRNTVDPTVKNYQWGDLTAASFEAKDRGARTAILLDADNCVAEGPGFNVVMVKDGKLSSPSRNALPGITRLTVMEMADEMGIEFTLRDITSRELYEADELIAVTTGGGITPITSLDGEPLGDGTPGPVTVAIRDRFWAMMDEPSSLVEAIEY

SEQ ID NO: 5 - protein, 341 aa, (Actinobacteria sp.)
MTISKDIDYSTSNLVSVAPGAIREPTPAGSVIQYSDYELDESSPFAGGAAWIEGEYVPAAEARISLFDTGFGHSDLTYTVAHVWHGNIFRLKDHINRVFDGAQILRLQSPLTKAEVEDITKRCVSLSQLRESFVNITITRGYGARKGEKDLSKLTSQIYIYAIPYLWAFPPEEQIFGTSAIVPRHVRRAGRNTVDPTVKNYQWGDLTAASFEAKDRGARTAILLDADNCVAEGPGFNVVMVKDGKLSSPSRNALPGITRLTVMEMADEMGIEFTLRDITSRELYEADELIAVTTGGGITPITSLDGEPLGDGTPGPVTVAIRDRFWAMMDEPSSLVEAIEY

SEQ ID NO: 6 - protein, 341 aa, (Actinobacteria sp.)
MTISKDIDYSTSNLVSVAPGAIREPTPAGSVIQYSDYELDESSPFAGGAAWIEGEYVPAAEARISLFDTGFGHSDATYTVAHVWHGNIFRLKDHIDRVFDGAQKLRLQSPLTKAEVEDITKRCVALSQLRESFVNITITRGYGARKGEKDLSKLTSQIYIYAIPYLWAFPPEEQIFGTSAIVPRHVRRAGRNTVDPTVKNYQWGDLTAASFEAKDRGARTAILLDGDNCVAEGPGFNVVMVKDGKLSSPSRNALPGITRLTVMEMADEMGIEFTLRDITSRELYEADELIAVTTGGGITPITSLDGEPLGDGTPGPVTVAIRDRFWAMMDEPSSLVEAIEY

SEQ ID NO: 7 - protein, 341 aa, (Actinobacteria sp.)
MTISKDIDYSTSNLVSVAPGAIREPTPAGSVIQYSDYELDESSPFAGGAAWIEGEYVPAAEARISLFDTGFGHSDATYTVAHVWHGNIFRLKDHIDRVFDGAQKLRLQSPLTKAEVEDITKRCVALSQLREAFVNITITRGYGARKGEKDLSKLTSQIYIYAIPYLWAFPPEEQIFGTSAIVPRHVRRAGRNTVDPTVKNYQWGDLTAASFEAKDRGARTAILLDGDNCVAEGPGFNVVMVKDGKLSSPSRNALPGITRLTVMEMADEMGIEFTLRDITSRELYEADELIAVTTGGGITPITSLDGEPLGDGTPGPVTVAIRDRFWAMMDEPSSLVEAIEY

SEQ ID NO: 8 - protein, 341 aa, (Actinobacteria sp.)
MTISKDIDYSTSNLVSVAPGAIREPTPAGSVIQYSDYELDESSPFAGGAAWIEGEYVPAAEARISLFDTGFGHSDLTYTVAHVWHGNIFRLKDHIDRVFDGAQKLRLQSPLTKAEVEDITKRCVSLSQLREAFVNITITRGYGARKGEKDLSKLTSQIYIYAIPYLWAFPPEEQIFGTSAIVPRHVRRAGRNTVDPTVKNYQWGDLTAASFEAKDRGARTAILLDADNCVAEGPGFNVVMVKDGKLSSPSRNALPGITRLTVMEMADEMGIEFTLRDITSRELYEADELIAVTTGGGITPITSLDGEPLGDGTPGPVTVAIRDRFWAMMDEPSSLVEAIEY

SEQ ID NO: 9 - protein, 341 aa, (Actinobacteria sp.)
MTISKDIDYSTSNLVSVAPGAIREPTPAGSVIQYSDYELDESSPFAGGAAWIEGEYVPAAEARISLFDTGFLHSDLTYTVAHVWHGNIFRLKDHIDRVFDGAQKLRLQSPLTKAEVEDITKRCVSLSQLRESFVNITITRGYGARKGEKDLSKLTSQIYIYAIPYLWAFPPEEQIFGTSAIVPRHVRRAGRNTVDPTVKNYQWGDLTAASFEAKDRGARTAILLDADNCVAEGPGFNVVMVKDGKLSSPSRNALPGITRLTVMEMADEMGIEFTLRDITSRELYEADELIAVTTGGGITPITSLDGEPLGDGTPGPVTVAIRDRFWAMMDEPSSLVEAIEY

SEQ ID NO: 10 - protein, 341 aa, (Actinobacteria sp.)
MTISKDIDYSTSNLVSVAPGAIREPTPAGSVIQYSDYELDESSPFAGGAAWIEGEYVPAAEARISLFDTGFLHSDLTYTVAHVWHGNIFRLKDHIDRVFDGAQKLRLQSPLTKAEVEDITKRCVSLSQLREAFVNITITRGYGARKGEKDLSKLTSQIYIYAIPYLWAFPPEEQIFGTSAIVPRHVRRAGRNTVDPTVKNYQWGDLTAASFEAKDRGARTAILLDADNCVAEGPGFNVVMVKDGKLSSPSRNALPGITRLTVMEMADEMGIEFTLRDITSRELYEADELIAVTTGGGITPITSLDGEPLGDGTPGPVTVAIRDRFWAMMDEPSSLVEAIEY

SEQ ID NO: 11 - protein, 341 aa, (Actinobacteria sp.)
MTISKDIDYSTSNLVSVAPGAIREPTPAGSVIQYSDYELDESSPFAGGAAWIEGEYVPAAEARISLFDTGFLHSDLTYTVAHVWHGNIFRLKDHIDRVFDGAQKLRLQSPLTKAEVEDITKRCVSLSQLRESFVNITITRGYGARKGEKDLSKLTSQIYIYAIPYLWAFPPEEQIFGTSAIVPRHVRRAGRNTVDPTVKNYQWGDLTAASFEAKDRGARTAILLDADNCVAEGPGFNVVMVKDGKLSSPSRNALPGITRLTVMEMADEMGIEFTLRDITSRELYEADELIACTTGGGITPITSLDGEPLGDGTPGPVTVAIRDRFWAMMDEPSSLVEAIEY

SEQ ID NO: 12 - protein, 341 aa, (Actinobacteria sp.)
MTISKDIDYSTSNLVSVAPGAIREPTPAGSVIQYSDYELDESSPFAGGAAWIEGEYVPAAEARISLFDTGFLHSDATYTVAHVWHGNIFRLKDHIDRVFDGAQKLRLQSPLTKAEVEDITKRCVSLSQLRESFVNITITRGYGARKGEKDLSKLTSQIYIYAIPYLWAFPPEEQIFGTSAIVPRHVRRAGRNTVDPTVKNYQWGDLTAASFEAKDRGARTAILLDADNCVAEGPGFNVVMVKDGKLSSPSRNALPGITRLTVMEMADEMGIEFTLRDITSRELYEADELIACTTGGGITPITSLDGEPLGDGTPGPVTVAIRDRFWAMMDEPSSLVEAIEY

SEQ ID NO: 13 - protein, 341 aa, (Actinobacteria sp.)
MTISKDIDYSTSNLVSVAPGAIREPTPAGSVIQYSDYELDESSPFAGGAAWIEGEYVPAAEARISLFDTGFLHSDLTYTVAHVWHGNIFRLKDHIDRVFDGAQKLRLQSPLTKAEVEDITKRCVSLSQLRESFVNITITRGYGARKGEKDLSKLTSQIYIYAIPYLWAFPPEEQIFGTSAIVPRHVRRAGRNTVDPTVKNYQWGDLTAASFEAKDRGARTAILLDADNCVAEGPGFNVVMVKDGKLSSPSRNALPGITRLTVMEMADEMGIEFTLRDITSRELYEADELIAVTTAGGITPITSLDGEPLGDGTPGPVTVAIRDRFWAMMDEPSSLVEAIEY

SEQ ID NO: 14 - protein, 341 aa, (Actinobacteria sp.)
MTISKDIDYSTSNLVSVAPGAIREPTPAGSVIQYSDYELDESSPFAGGAAWIEGEYVPAAEARISLFDTGFGHSDATYTVAHVWHGNIFRLKDHIDRVFDGAQKLRLQSPLTKAEVEDITKRCVSLSQLRESFVNITITRGYGARKGEKDLSKLTSQIYIYAIPYLWAFPPEEQIFGTSAIVPRHVRRAGRNTVDPTVKNYQWGDLTAASFEAKDRGARTAILLDADNCVAEGPGFNVVMVKDGKLSSPSRNALPGITRLTVMEMADEMGIEFTLRDITSRELYEADELIAVTTAGGITPITSLDGEPLGDGTPGPVTVAIRDRFWAMMDEPSSLVEAIEY

SEQ ID NO: 15 - protein, 341 aa, (Actinobacteria sp.)
MTISKDIDYSTSNLVSVAPGAIREPTPAGSVIQYSDYELDESSPFAGGAAWIEGEYVPAAEARISLFDTGFGHSDLTYTVAHVWHGNIFRLKDHIDRVFDGAQKLRIQSPLTKAEVEDITKRCVSLSQLRESFVNITITRGYGARKGEKDLSKLTSQIYIYAIPYLWAFPPEEQIFGTSAIVPRHVRRAGRNTVDPTVKNYQWGDLTAASFEAKDRGARTAILLDADNCVAEGPGFNVVMVKDGKLSSPSRNALPGITRLTVMEMADEMGIEFTLRDITSRELYEADELIAVTTAGGITPITSLDGEPLGDGTPGPVTVAIRDRFWAMMDEPSSLVEAIEY

SEQ ID NO: 16 - protein, 341 aa, (Actinobacteria sp.)
MTISKDIDYSTSNLVSVAPGAIREPTPAGSVIQYSDYELDESSPFAGGAAWIEGEYVPAAEARISLFDTGFGHSDLTYTVAHVWHGNIFRLGDHIDRVFDGAQKLRLQSPLTKAEVEDITKRCVSLSQLRESFVNITITRGYGARKGEKDLSKLTSQIYIYAIPYLWAFPPEEQIFGTSAIVPRHVRRAGRNTVDPTVKNYQWGDLTAASFEAKDRGARTAILLDADNCVAEGPGFNVVMVKDGKLSSPSRNALPGITRLTVMEMADEMGIEFTLRDITSRELYEADELIAVTTAGGITPITSLDGEPLGDGTPGPVTVAIRDRFWAMMDEPSSLVEAIEY

SEQ ID NO: 17 - protein, 341 aa, (Actinobacteria sp.)
MTISKDIDYSTSNLVSVAPGAIREPTPAGSVIQYSDYELDESSPFAGGAAWIEGEYVPAAEARISLFDTGFGHSDLTYTVAHVWHGNIFRLKDHIDRVFDGAQKLRLQSPLTKAEVEDITKRCVALSQLRESFVNITITRGYGARKGEKDLSKLTSQIYIYAIPYLWAFPPEEQIFGTSAIVPRHVRRAGRNTVDPTVKNYQWGDLTAASFEAKDRGARTAILLDADNCVAEGPGFNVVMVKDGKLSSPSRNALPGITRLTVMEMADEMGIEFTLRDITSRELYEADELIAVTTAGGITPITSLDGEPLGDGTPGPVTVAIRDRFWAMMDEPSSLVEAIEY

SEQ ID NO: 18 - protein, 341 aa, (Actinobacteria sp.)
MTISKDIDYSTSNLVSVAPGAIREPTPAGSVIQYSDYELDESSPFAGGAAWIEGEYVPAAEARISLFDTGFGHSDLTYTVAHVWHGNIFRLKDHIDRVFDGAQKLRLQSPLTKAEVEDITKRCVSLSQLREAFVNITITRGYGARKGEKDLSKLTSQIYIYAIPYLWAFPPEEQIFGTSAIVPRHVRRAGRNTVDPTVKNYQWGDLTAASFEAKDRGARTAILLDADNCVAEGPGFNVVMVKDGKLSSPSRNALPGITRLTVMEMADEMGIEFTLRDITSRELYEADELIAVTTAGGITPITSLDGEPLGDGTPGPVTVAIRDRFWAMMDEPSSLVEAIEY

SEQ ID NO: 19 - protein, 341 aa, (Actinobacteria sp.)
MTISKDIDYSTSNLVSVAPGAIREPTPAGSVIQYSDYELDESSPFAGGAAWIEGEYVPAAEARISLFDTGFGHSDLTYTVAHVWHGNIFRLKDHIDRVFDGAQKLRLQSPLTKAEVEDITKRCVSLSQLRESFVNITITRGYGARKGEKDLSKLTSQIYIYAIPYLWAFPPEEQIFGTSAIVPRHVRRAGRNTVDPTVKNYQWGDLTAASFEAKDRGARTAILLDGDNCVAEGPGFNVVMVKDGKLSSPSRNALPGITRLTVMEMADEMGIEFTLRDITSRELYEADELIAVTTAGGITPITSLDGEPLGDGTPGPVTVAIRDRFWAMMDEPSSLVEAIEY

SEQ ID NO: 20 - protein, 341 aa, (Actinobacteria sp.)
MTISKDIDYSTSNLVSVAPGAIREPTPAGSVIQYSDYELDESSPFAGGAAWIEGEYVPAAEARISLFDTGFGHSDLTYTVAHVWHGNIFRLKDHIDRVFDGAQKLRLQSPLTKAEVEDITKRCVSLSQLRESFVNITITRGYGARKGEKDLSKLTSQIYIYAIPYLWAFPPEEQIFGTSAIVPRHVRRAGRNTVDPTVKNYQWGDLTAASFEAKDRGARTAILLDADNCVAEGPGFNVVMVKDGKLSSPSRNALPGITRLTVMEMADEMGIEFTLRDITSRELYEADELIACTTAGGITPITSLDGEPLGDGTPGPVTVAIRDRFWAMMDEPSSLVEAIEY

SEQ ID NO: 21 - protein, 341 aa, (Actinobacteria sp.)
MTISKDIDYSTSNLVSVAPGAIREPTPAGSVIQYSDYELDESSPFAGGAAWIEGEYVPAAEARISLFDTGFGHSDLTYTVAHVWHGNIFRLKDHIDRVFDGAQKLRLQSPLTKAEVEDITKRCVSLSQLRESFVNITITRGYGARKGEKDLSKLTSQIYIYAIPYLWAFPPEEQIFGTSAIVPRHVRRAGRNTVDPTVKNYQWGDLTAASFEAKDRGARTAILLDADNCVAEGPGFNVVMVKDGKLSSPSRNALPGITRLTVMEMADEMGIEFTLRDITSRELYEADELIAVTTGGGITPITSLDGEPLGDGTPGPVTVAIRDRFWAMMDEPSSLVEAIEY

SEQ ID NO: 22 - protein, 341 aa, (Actinobacteria sp.)
MTISKDIDYSTSNLVSVASGAIREPTPAGSVIQYSDYELDESSPFAGGAAWIEGEYVPAAEARISLFDTGFGHSDLTYTVAHVWHGNIFRLKDHIDRVFDGAQKLRLQSPLTKAEVEDITKRCVSLSQLRESFVNITITRGYGARKGEKDLSKLTSQIYIYAIPYLWAFPPEEQIFGTSAIVPRHVRRAGRNTVDPTVKNYQWGDLTAASFEAKDRGARTAILLDADNCVAEGPGFNVVMVKDGKLSSPSRNALPGITRLTVMEMADEMGIEFTLRDITSRELYEADELIAVTTAGGITPITSLDGEPLGDGTPGPVTVAIRDRFWAMMDEPSSLVEAIEY

SEQ ID NO: 23 - protein, 341 aa, (Actinobacteria sp.)
MTISKDIDYSTSNLVSVAPGAIREPTPAGSVIQYSDYELDSSSPFAGGAAWIEGEYVPAAEARISLFDTGFGHSDLTYTVAHVWHGNIFRLKDHIDRVFDGAQKLRLQSPLTKAEVEDITKRCVSLSQLRESFVNITITRGYGARKGEKDLSKLTSQIYIYAIPYLWAFPPEEQIFGTSAIVPRHVRRAGRNTVDPTVKNYQWGDLTAASFEAKDRGARTAILLDADNCVAEGPGFNVVMVKDGKLSSPSRNALPGITRLTVMEMADEMGIEFTLRDITSRELYEADELIAVTTAGGITPITSLDGEPLGDGTPGPVTVAIRDRFWAMMDEPSSLVEAIEY

SEQ ID NO: 24 - protein, 341 aa, (Actinobacteria sp.)
MTISKDIDYSTSNLVSVAPGAIREPTPAGSVIQYSDYELDESNPFAGGAAWIEGEYVPAAEARISLFDTGFGHSDLTYTVAHVWHGNIFRLKDHIDRVFDGAQKLRLQSPLTKAEVEDITKRCVSLSQLRESFVNITITRGYGARKGEKDLSKLTSQIYIYAIPYLWAFPPEEQIFGTSAIVPRHVRRAGRNTVDPTVKNYQWGDLTAASFEAKDRGARTAILLDADNCVAEGPGFNVVMVKDGKLSSPSRNALPGITRLTVMEMADEMGIEFTLRDITSRELYEADELIAVTTAGGITPITSLDGEPLGDGTPGPVTVAIRDRFWAMMDEPSSLVEAIEY

SEQ ID NO: 25 - protein, 341 aa, (Actinobacteria sp.)
MTISKDIDYSTSNLVSVAPGAIREPTPAGSVIQYSDYELDESSPFAGGAAWIEGEYVPAAEARISLFDTGFGHSDLTYTVAHVWHGNIFRLKDHIDRVFDGAQKLRLQSPLTKAEVEDITKRCVSLSQLRESFVNITITRGYGARKGEKDLSKLTSQIYIYAIPYLWAFPPEEQIFGTSAIVPRHVRRAGRNTVDPTVKNYQWGDLTAASFEAKDRGARTAILLDADNCVAEGPGFNVVMVKDGKLSSPSRNALPGITRLTVMEMADEMGIEFTLRDITSRELYEADELIAVTTAGGITPITSLDGESLGDGTPGPVTVAIRDRFWAMMDEPSSLVEAIEY

SEQ ID NO: 26 - protein, 341 aa, (Actinobacteria sp.)
MTISKDIDYSTSNLVSVAPGAIREPTPAGSVIQYSDYELDESSPFAGGAAWIEGEYVPAAEARISLFDTGFGHSDLTYTVAHVWHGNIFRLKDHIDRVFDGAQKLRLQSPLTKAEVEDITKRCVSLSQLRESFVNITITRGYGARKGEKDLSKLTSQIYIYAIPYLWAFPPEEQIFGTSAIVPRHVRRAGRNTVDPTVKNYQWGDLTAASFEAKDRGARTAILLDADNCVAEGPGFNVVMVKDGKLSSPSRNALPGITRLTVMEMADEMGIEFTLRDITSRELYEADELIAVTTAGGITPITSLDGEPLGDGTPGPVTVAIRDRFWAMMDESSSLVEAIEY

SEQ ID NO: 27 - protein, 341 aa, (Actinobacteria sp.)
MTISKDIDYSTSNLVSVAPGAIREPTPAGSVIQYSDYELDESSPFAGGAAWIEGEYVPAAEARISLFDTGFGHSDATYTVAHVWHGNIFRLKDHIDRVFDGAQKLRIQSQLTKAEVEDITKRCVSLSQLRESFVNITITRGYGARKGEKDLSKLTSQIYIYAIPYLWAFPPEEQIFGTSAIVPRHVRRAGRNTVDPTVKNYQWGDLTAASFEAKDRGARTAILLDADNCVAEGPGFNVVMVKDGKLSSPSRNALPGITRLTVMEMADEMGIEFTLRDITSRELYEADELIAVTTAGGITPITSLDGEPLGDGTPGPVTVAIRDRFWAMMDEPSSLVEAIEY

SEQ ID NO: 28 - protein, 341 aa, (Actinobacteria sp.)
MTISKDIDYSTSNLVSVAPGAIREPTPAGSVIQYSDYELDESSPFAGGAAWIEGEYVPAAEARISLFDTGFGHSDATYTVAHVWHGNIFRLKDHIDRVFDGAQKLRLQSPLTKAEVEDITKRCVALSQLRESFVNITITRGYGARKGEKDLSKLTSQIYIYAIPYLWAFPPEEQIFGTSAIVPRHVRRAGRNTVDPTVKNYQWGDLTAASFEAKDRGARTAILLDGDNCVAEGPGFNVVMVKDGKLSSPSRNALPGITRLTVMEMADEMGIEFTLRDITSRELYEADELIAVTTAGGITPITSLDGEPLGDGTPGPVTVAIRDRFWAMMDEPSSLVEAIEY

SEQ ID NO: 29 - protein, 341 aa, (Actinobacteria sp.)
MTISKDIDYSTSNLVSVAPGAIREPTPAGSVIQYSDYELDESSPFAGGAAWIEGEYVPAAEARISLFDTGFGHSDATYSVAHVWHGNIFRLKDHIDRVFDGAQKLRLQSPLTKAEVEDITKRCVSLSQLRESFVNITITRGYGARKGEKDLSKLTSQIYIYAIPYLWAFPPEEQIFGTSAIVPRHVRRAGRNTVDPTVKNYQWGDLTAASFEAKDRGARTAILLDADNCVAEGPGFNVVMVKDGKLSSPSRNALPGITRLTVMEMADEMGIEFTLRDITSRELYEADELIAVTTGGGITPITSLDGEPLGDGTPGPVTVAIRDRFWAMMDEPSSLVEAIEY

SEQ ID NO: 30 - protein, 341 aa, (Actinobacteria sp.)
MTISKDIDYSTSNLVSVAPGAIREPTPAGSVIQYSDYELDESSPFAGGAAWIEGEYVPAAEARISLFDTGFGHSDATYTVAHVWHGNIFRLKDHIDRVFDGAQKLRIQSQLTKAEVEDITKRCVSLSQLRESFVNITITRGYGARKGEKGLSKLTSQIYIYAIPYLWAFPPEEQIFGTSAIVPRHVRRAGRNTVDPTVKNYQWGDLTAASFEAKDRGARTAILLDADNCVAEGPGFNVVMVKDGKLSSPSRNALPGITRLTVMEMADEMGIEFTLRDITSRELYEADELIAVTTAGGITPITSLDGEPLGDGTPGPVTVAIRDRFWAMMDEPSSLVEAIEY

SEQ ID NO: 31 - DNA, 1026 bp, (Actinobacteria sp.)
atgaccattagcaaagacattgactatagcaccagcaacctggtgagtgtggccccgggtgcaatccgtgaacctaccccggcaggcagcgtgatccagtacagtgactacgagctggatgaaagcagcccgtttgccggtggtgcagcctggattgaaggtgagtatgttccggcagcagaggcccgtattagcctgtttgataccggcttcggccatagcgatctgacctacaccgttgcccatgtttggcacggcaacatctttcgcctgaaagaccacattgaccgcgtgtttgatggcgcccagaaactgcgtctgcagagcccgctgaccaaggccgaagtggaggatattaccaaacgctgcgtgagcctgagtcagctgcgcgagagcttcgtgaacatcaccattacccgcggttatggcgcccgcaaaggcgagaaagatctgagcaaattaaccagccagatctacatctacgccatcccgtacctgtgggcctttcctccggaagagcagatcttcggtacaagtgccattgtgccgcgtcatgttcgtcgcgcaggccgtaataccgttgatcctaccgttaagaactaccagtggggtgatctgaccgcagcttcttttgaagcaaaagatcgtggcgcccgcaccgcaatcctgctggatgcagacaactgtgtggccgagggtccgggctttaacgtggtgatggtgaaggatggcaaactgagtagcccgagccgtaatgccctgccgggtattacacgtctgaccgtgatggagatggccgatgaaatgggcatcgaattcaccctgcgcgatatcaccagccgtgagttatatgaggccgacgaactgatcgccgtgaccaccgcaggtggcattaccccgattaccagtctggatggcgaaccgctgggcgatggtacccctggtcctgtgacagtggccattcgcgatcgcttttgggccatgatggatgagccgagcagtctggtggaggccattgaatattaa

SEQ ID NO: 32 - DNA, 1026 bp, (Actinobacteria sp.)
atgaccattagcaaagacattgactatagcaccagcaacctggtgagtgtggccccgggtgcaatccgtgaacctaccccggcaggcagcgtgatccagtacagtgactacgagctggatgaaagcagcccgtttgccggtggtgcagcctggattgaaggtgagtatgttccggcagcagaggcccgtattagcctgtttgataccggcttcggccatagcgatgcgacctacaccgttgcccatgtttggcacggcaacatctttcgcctgaaagaccacattgaccgcgtgtttgatggcgcccagaaactgcgtctgcagagcccgctgaccaaggccgaagtggaggatattaccaaacgctgcgtgagcctgagtcagctggccgagagcttcgtgaacatcaccattacccgcggttatggcgcccgcaaaggcgagaaagatctgagcaaattaaccagccagatctacatctacgccatcccgtacctgtgggcctttcctccggaagagcagatcttcggtacaagtgccattgtgccgcgtcatgttcgtcgcgcaggccgtaataccgttgatcctaccgttaagaactaccagtggggtgatctgaccgcagcttcttttgaagcaaaagatcgtggcgcccgcaccgcaatcctgctggatgcagacaactgtgtggccgagggtccgggctttaacgtggtgatggtgaaggatggcaaactgagtagcccgagccgtaatgccctgccgggtattacacgtctgaccgtgatggagatggccgatgaaatgggcatcgaattcaccctgcgcgatatcaccagccgtgagttatatgaggccgacgaactgatcgcctgcaccaccggaggtggcattaccccgattaccagtctggatggcgaaccgctgggcgatggtacccctggtcctgtgacagtggccattcgcgatcgcttttgggccatgatggatgagccgagcagtctggtggaggccattgaatattaa

SEQ ID NO: 33 - DNA, 1026 bp, (Actinobacteria sp.)
atgaccattagcaaagacattgactatagcaccagcaacctggtgagtgtggccccgggtgcaatccgtgaacctaccccggcaggcagcgtgatccagtacagtgactacgagctggatgaaagcagcccgtttgccggtggtgcagcctggattgaaggtgagtatgttccggcagcagaggcccgtattagcctgtttgataccggcttcggccatagcgatctgacctacaccgttgcccatgtttggcacggcaacatctttcgcctgaaagaccacattgaccgcgtgtttgatggcgcccagaaactgcgtatacagagcccgctgaccaaggccgaagtggaggatattaccaaacgctgcgtgagcctgagtcagctgcgcgagagcttcgtgaacatcaccattacccgcggttatggcgcccgcaaaggcgagaaagatctgagcaaattaaccagccagatctacatctacgccatcccgtacctgtgggcctttcctccggaagagcagatcttcggtacaagtgccattgtgccgcgtcatgttcgtcgcgcaggccgtaataccgttgatcctaccgttaagaactaccagtggggtgatctgaccgcagcttcttttgaagcaaaagatcgtggcgcccgcaccgcaatcctgctggatgcagacaactgtgtggccgagggtccgggctttaacgtggtgatggtgaaggatggcaaactgagtagcccgagccgtaatgccctgccgggtattacacgtctgaccgtgatggagatggccgatgaaatgggcatcgaattcaccctgcgcgatatcaccagccgtgagttatatgaggccgacgaactgatcgccgtgaccaccggaggtggcattaccccgattaccagtctggatggcgaaccgctgggcgatggtacccctggtcctgtgacagtggccattcgcgatcgcttttgggccatgatggatgagccgagcagtctggtggaggccattgaatattaa

SEQ ID NO: 34 - DNA, 1026 bp, (Actinobacteria sp.)
atgaccattagcaaagacattgactatagcaccagcaacctggtgagtgtggccccgggtgcaatccgtgaacctaccccggcaggcagcgtgatccagtacagtgactacgagctggatgaaagcaacccgtttgccggtggtgcagcctggattgaaggtgagtatgttccggcagcagaggcccgtattagcctgtttgataccggcttcctacatagcgatctgacctacaccgttgcccatgtttggcacggcaacatctttcgcctgaaagaccacattgaccgcgtgtttgatggcgcccagaaactgcgtctgcagagcccgctgaccaaggccgaagtggaggatattaccaaacgctgcgtgagcctgagtcagctgcgcgagagcttcgtgaacatcaccattacccgcggttatggcgcccgcaaaggcgagaaagatctgagcaaattaaccagccagatctacatctacgccatcccgtacctgtgggcctttcctccggaagagcagatcttcggtacaagtgccattgtgccgcgtcatgttcgtcgcgcaggccgtaataccgttgatcctaccgttaagaactaccagtggggtgatctgaccgcagcttcttttgaagcaaaagatcgtggcgcccgcaccgcaatcctgctggatgcagacaactgtgtggccgagggtccgggctttaacgtggtgatggtgaaggatggcaaactgagtagcccgagccgtaatgccctgccgggtattacacgtctgaccgtgatggagatggccgatgaaatgggcatcgaattcaccctgcgcgatatcaccagccgtgagttatatgaggccgacgaactgatcgccgtgaccaccggaggtggcattaccccgattaccagtctggatggcgaaccgctgggcgatggtacccctggtcctgtgacagtggccattcgcgatcgcttttgggccatgatggatgagccgagcagtctggtggaggccattgaatattaa

SEQ ID NO: 35 - DNA, 1026 bp, (Actinobacteria sp.)
atgaccattagcaaagacattgactatagcaccagcaacctggtgagtgtggccccgggtgcaatccgtgaacctaccccggcaggcagcgtgatccagtacagtgactacgagctggatgaaagcagcccgtttgccggtggtgcagcctggattgaaggtgagtatgttccggcagcagaggcccgtattagcctgtttgataccggcttcggccatagcgatctgacctacaccgttgcccatgtttggcacggcaacatctttcgcctgaaagaccacattaaccgcgtgtttgatggcgcccagatactgcgtctgcagagcccgctgaccaaggccgaagtggaggatattaccaaacgctgcgtgagcctgagtcagctgcgcgagagcttcgtgaacatcaccattacccgcggttatggcgcccgcaaaggcgagaaagatctgagcaaattaaccagccagatctacatctacgccatcccgtacctgtgggcctttcctccggaagagcagatcttcggtacaagtgccattgtgccgcgtcatgttcgtcgcgcaggccgtaataccgttgatcctaccgttaagaactaccagtggggtgatctgaccgcagcttcttttgaagcaaaagatcgtggcgcccgcaccgcaatcctgctggatgcagacaactgtgtggccgagggtccgggctttaacgtggtgatggtgaaggatggcaaactgagtagcccgagccgtaatgccctgccgggtattacacgtctgaccgtgatggagatggccgatgaaatgggcatcgaattcaccctgcgcgatatcaccagccgtgagttatatgaggccgacgaactgatcgccgtgaccaccggaggtggcattaccccgattaccagtctggatggcgaaccgctgggcgatggtacccctggtcctgtgacagtggccattcgcgatcgcttttgggccatgatggatgagccgagcagtctggtggaggccattgaatattaa

SEQ ID NO: 36 - DNA, 1026 bp, (Actinobacteria sp.)
atgaccattagcaaagacattgactatagcaccagcaacctggtgagtgtggccccgggtgcaatccgtgaacctaccccggcaggcagcgtgatccagtacagtgactacgagctggatgaaagcagcccgtttgccggtggtgcagcctggattgaaggtgagtatgttccggcagcagaggcccgtattagcctgtttgataccggcttcggccatagcgatgcgacctacaccgttgcccatgtttggcacggcaacatctttcgcctgaaagaccacattgaccgcgtgtttgatggcgcccagaaactgcgtctgcagagcccgctgaccaaggccgaagtggaggatattaccaaacgctgcgtggccctgagtcagctgcgcgagagcttcgtgaacatcaccattacccgcggttatggcgcccgcaaaggcgagaaagatctgagcaaattaaccagccagatctacatctacgccatcccgtacctgtgggcctttcctccggaagagcagatcttcggtacaagtgccattgtgccgcgtcatgttcgtcgcgcaggccgtaataccgttgatcctaccgttaagaactaccagtggggtgatctgaccgcagcttcttttgaagcaaaagatcgtggcgcccgcaccgcaatcctgctggatgcggacaactgtgtggccgagggtccgggctttaacgtggtgatggtgaaggatggcaaactgagtagcccgagccgtaatgccctgccgggtattacacgtctgaccgtgatggagatggccgatgaaatgggcatcgaattcaccctgcgcgatatcaccagccgtgagttatatgaggccgacgaactgatcgccgtgaccaccggaggtggcattaccccgattaccagtctggatggcgaaccgctgggcgatggtacccctggtcctgtgacagtggccattcgcgatcgcttttgggccatgatggatgagccgagcagtctggtggaggccattgaatattaa

SEQ ID NO: 37 - DNA, 1026 bp, (Actinobacteria sp.)
atgaccattagcaaagacattgactatagcaccagcaacctggtgagtgtggccccgggtgcaatccgtgaacctaccccggcaggcagcgtgatccagtacagtgactacgagctggatgaaagcagcccgtttgccggtggtgcagcctggattgaaggtgagtatgttccggcagcagaggcccgtattagcctgtttgataccggcttcggccatagcgatgcgacctacaccgttgcccatgtttggcacggcaacatctttcgcctgaaagaccacattgaccgcgtgtttgatggcgcccagaaactgcgtctgcagagcccgctgaccaaggccgaagtggaggatattaccaaacgctgcgtggccctgagtcagctgcgcgaggccttcgtgaacatcaccattacccgcggttatggcgcccgcaaaggcgagaaagatctgagcaaattaaccagccagatctacatctacgccatcccgtacctgtgggcctttcctccggaagagcagatcttcggtacaagtgccattgtgccgcgtcatgttcgtcgcgcaggccgtaataccgttgatcctaccgttaagaactaccagtggggtgatctgaccgcagcttcttttgaagcaaaagatcgtggcgcccgcaccgcaatcctgctggatgcggacaactgtgtggccgagggtccgggctttaacgtggtgatggtgaaggatggcaaactgagtagcccgagccgtaatgccctgccgggtattacacgtctgaccgtgatggagatggccgatgaaatgggcatcgaattcaccctgcgcgatatcaccagccgtgagttatatgaggccgacgaactgatcgccgtgaccaccggaggtggcattaccccgattaccagtctggatggcgaaccgctgggcgatggtacccctggtcctgtgacagtggccattcgcgatcgcttttgggccatgatggatgagccgagcagtctggtggaggccattgaatattaa

SEQ ID NO: 38 - DNA, 1026 bp, (Actinobacteria sp.)
atgaccattagcaaagacattgactatagcaccagcaacctggtgagtgtggccccgggtgcaatccgtgaacctaccccggcaggcagcgtgatccagtacagtgactacgagctggatgaaagcagcccgtttgccggtggtgcagcctggattgaaggtgagtatgttccggcagcagaggcccgtattagcctgtttgataccggcttcggccatagcgatctgacctacaccgttgcccatgtttggcacggcaacatctttcgcctgaaagaccacattgaccgcgtgtttgatggcgcccagaaactgcgtctgcagagcccgctgaccaaggccgaagtggaggatattaccaaacgctgcgtgagcctgagtcagctgcgcgaggccttcgtgaacatcaccattacccgcggttatggcgcccgcaaaggcgagaaagatctgagcaaattaaccagccagatctacatctacgccatcccgtacctgtgggcctttcctccggaagagcagatcttcggtacaagtgccattgtgccgcgtcatgttcgtcgcgcaggccgtaataccgttgatcctaccgttaagaactaccagtggggtgatctgaccgcagcttcttttgaagcaaaagatcgtggcgcccgcaccgcaatcctgctggatgcagacaactgtgtggccgagggtccgggctttaacgtggtgatggtgaaggatggcaaactgagtagcccgagccgtaatgccctgccgggtattacacgtctgaccgtgatggagatggccgatgaaatgggcatcgaattcaccctgcgcgatatcaccagccgtgagttatatgaggccgacgaactgatcgccgtgaccaccggaggtggcattaccccgattaccagtctggatggcgaaccgctgggcgatggtacccctggtcctgtgacagtggccattcgcgatcgcttttgggccatgatggatgagccgagcagtctggtggaggccattgaatattaa

SEQ ID NO: 39 - DNA, 1026 bp, (Actinobacteria sp.)
atgaccattagcaaagacattgactatagcaccagcaacctggtgagtgtggccccgggtgcaatccgtgaacctaccccggcaggcagcgtgatccagtacagtgactacgagctggatgaaagcagcccgtttgccggtggtgcagcctggattgaaggtgagtatgttccggcagcagaggcccgtattagcctgtttgataccggcttcctacatagcgatctgacctacaccgttgcccatgtttggcacggcaacatctttcgcctgaaagaccacattgaccgcgtgtttgatggcgcccagaaactgcgtctgcagagcccgctgaccaaggccgaagtggaggatattaccaaacgctgcgtgagcctgagtcagctgcgcgagagcttcgtgaacatcaccattacccgcggttatggcgcccgcaaaggcgagaaagatctgagcaaattaaccagccagatctacatctacgccatcccgtacctgtgggcctttcctccggaagagcagatcttcggtacaagtgccattgtgccgcgtcatgttcgtcgcgcaggccgtaataccgttgatcctaccgttaagaactaccagtggggtgatctgaccgcagcttcttttgaagcaaaagatcgtggcgcccgcaccgcaatcctgctggatgcagacaactgtgtggccgagggtccgggctttaacgtggtgatggtgaaggatggcaaactgagtagcccgagccgtaatgccctgccgggtattacacgtctgaccgtgatggagatggccgatgaaatgggcatcgaattcaccctgcgcgatatcaccagccgtgagttatatgaggccgacgaactgatcgccgtgaccaccggaggtggcattaccccgattaccagtctggatggcgaaccgctgggcgatggtacccctggtcctgtgacagtggccattcgcgatcgcttttgggccatgatggatgagccgagcagtctggtggaggccattgaatattaa

SEQ ID NO: 40 - DNA, 1026 bp, (Actinobacteria sp.)
atgaccattagcaaagacattgactatagcaccagcaacctggtgagtgtggccccgggtgcaatccgtgaacctaccccggcaggcagcgtgatccagtacagtgactacgagctggatgaaagcagcccgtttgccggtggtgcagcctggattgaaggtgagtatgttccggcagcagaggcccgtattagcctgtttgataccggcttcctacatagcgatctgacctacaccgttgcccatgtttggcacggcaacatctttcgcctgaaagaccacattgaccgcgtgtttgatggcgcccagaaactgcgtctgcagagcccgctgaccaaggccgaagtggaggatattaccaaacgctgcgtgagcctgagtcagctgcgcgaggccttcgtgaacatcaccattacccgcggttatggcgcccgcaaaggcgagaaagatctgagcaaattaaccagccagatctacatctacgccatcccgtacctgtgggcctttcctccggaagagcagatcttcggtacaagtgccattgtgccgcgtcatgttcgtcgcgcaggccgtaataccgttgatcctaccgttaagaactaccagtggggtgatctgaccgcagcttcttttgaagcaaaagatcgtggcgcccgcaccgcaatcctgctggatgcagacaactgtgtggccgagggtccgggctttaacgtggtgatggtgaaggatggcaaactgagtagcccgagccgtaatgccctgccgggtattacacgtctgaccgtgatggagatggccgatgaaatgggcatcgaattcaccctgcgcgatatcaccagccgtgagttatatgaggccgacgaactgatcgccgtgaccaccggaggtggcattaccccgattaccagtctggatggcgaaccgctgggcgatggtacccctggtcctgtgacagtggccattcgcgatcgcttttgggccatgatggatgagccgagcagtctggtggaggccattgaatattaa

SEQ ID NO: 41 - DNA, 1026 bp, (Actinobacteria sp.)
atgaccattagcaaagacattgactatagcaccagcaacctggtgagtgtggccccgggtgcaatccgtgaacctaccccggcaggcagcgtgatccagtacagtgactacgagctggatgaaagcagcccgtttgccggtggtgcagcctggattgaaggtgagtatgttccggcagcagaggcccgtattagcctgtttgataccggcttcctacatagcgatctgacctacaccgttgcccatgtttggcacggcaacatctttcgcctgaaagaccacattgaccgcgtgtttgatggcgcccagaaactgcgtctgcagagcccgctgaccaaggccgaagtggaggatattaccaaacgctgcgtgagcctgagtcagctgcgcgagagcttcgtgaacatcaccattacccgcggttatggcgcccgcaaaggcgagaaagatctgagcaaattaaccagccagatctacatctacgccatcccgtacctgtgggcctttcctccggaagagcagatcttcggtacaagtgccattgtgccgcgtcatgttcgtcgcgcaggccgtaataccgttgatcctaccgttaagaactaccagtggggtgatctgaccgcagcttcttttgaagcaaaagatcgtggcgcccgcaccgcaatcctgctggatgcagacaactgtgtggccgagggtccgggctttaacgtggtgatggtgaaggatggcaaactgagtagcccgagccgtaatgccctgccgggtattacacgtctgaccgtgatggagatggccgatgaaatgggcatcgaattcaccctgcgcgatatcaccagccgtgagttatatgaggccgacgaactgatcgcctgcaccaccggaggtggcattaccccgattaccagtctggatggcgaaccgctgggcgatggtacccctggtcctgtgacagtggccattcgcgatcgcttttgggccatgatggatgagccgagcagtctggtggaggccattgaatattaa

SEQ ID NO: 42 - DNA, 1026 bp, (Actinobacteria sp.)
atgaccattagcaaagacattgactatagcaccagcaacctggtgagtgtggccccgggtgcaatccgtgaacctaccccggcaggcagcgtgatccagtacagtgactacgagctggatgaaagcagcccgtttgccggtggtgcagcctggattgaaggtgagtatgttccggcagcagaggcccgtattagcctgtttgataccggcttcctacatagcgatgcgacctacaccgttgcccatgtttggcacggcaacatctttcgcctgaaagaccacattgaccgcgtgtttgatggcgcccagaaactgcgtctgcagagcccgctgaccaaggccgaagtggaggatattaccaaacgctgcgtgagcctgagtcagctgcgcgagagcttcgtgaacatcaccattacccgcggttatggcgcccgcaaaggcgagaaagatctgagcaaattaaccagccagatctacatctacgccatcccgtacctgtgggcctttcctccggaagagcagatcttcggtacaagtgccattgtgccgcgtcatgttcgtcgcgcaggccgtaataccgttgatcctaccgttaagaactaccagtggggtgatctgaccgcagcttcttttgaagcaaaagatcgtggcgcccgcaccgcaatcctgctggatgcagacaactgtgtggccgagggtccgggctttaacgtggtgatggtgaaggatggcaaactgagtagcccgagccgtaatgccctgccgggtattacacgtctgaccgtgatggagatggccgatgaaatgggcatcgaattcaccctgcgcgatatcaccagccgtgagttatatgaggccgacgaactgatcgcctgcaccaccggaggtggcattaccccgattaccagtctggatggcgaaccgctgggcgatggtacccctggtcctgtgacagtggccattcgcgatcgcttttgggccatgatggatgagccgagcagtctggtggaggccattgaatattaa

SEQ ID NO: 43 - DNA, 1026 bp, (Actinobacteria sp.)
atgaccattagcaaagacattgactatagcaccagcaacctggtgagtgtggccccgggtgcaatccgtgaacctaccccggcaggcagcgtgatccagtacagtgactacgagctggatgaaagcagcccgtttgccggtggtgcagcctggattgaaggtgagtatgttccggcagcagaggcccgtattagcctgtttgataccggcttcctacatagcgatctgacctacaccgttgcccatgtttggcacggcaacatctttcgcctgaaagaccacattgaccgcgtgtttgatggcgcccagaaactgcgtctgcagagcccgctgaccaaggccgaagtggaggatattaccaaacgctgcgtgagcctgagtcagctgcgcgagagcttcgtgaacatcaccattacccgcggttatggcgcccgcaaaggcgagaaagatctgagcaaattaaccagccagatctacatctacgccatcccgtacctgtgggcctttcctccggaagagcagatcttcggtacaagtgccattgtgccgcgtcatgttcgtcgcgcaggccgtaataccgttgatcctaccgttaagaactaccagtggggtgatctgaccgcagcttcttttgaagcaaaagatcgtggcgcccgcaccgcaatcctgctggatgcagacaactgtgtggccgagggtccgggctttaacgtggtgatggtgaaggatggcaaactgagtagcccgagccgtaatgccctgccgggtattacacgtctgaccgtgatggagatggccgatgaaatgggcatcgaattcaccctgcgcgatatcaccagccgtgagttatatgaggccgacgaactgatcgccgtgaccaccgcaggtggcattaccccgattaccagtctggatggcgaaccgctgggcgatggtacccctggtcctgtgacagtggccattcgcgatcgcttttgggccatgatggatgagccgagcagtctggtggaggccattgaatattaa

SEQ ID NO: 44 - DNA, 1026 bp, (Actinobacteria sp.)
atgaccattagcaaagacattgactatagcaccagcaacctggtgagtgtggccccgggtgcaatccgtgaacctaccccggcaggcagcgtgatccagtacagtgactacgagctggatgaaagcagcccgtttgccggtggtgcagcctggattgaaggtgagtatgttccggcagcagaggcccgtattagcctgtttgataccggcttcggccatagcgatgcgacctacaccgttgcccatgtttggcacggcaacatctttcgcctgaaagaccacattgaccgcgtgtttgatggcgcccagaaactgcgtctgcagagcccgctgaccaaggccgaagtggaggatattaccaaacgctgcgtgagcctgagtcagctgcgcgagagcttcgtgaacatcaccattacccgcggttatggcgcccgcaaaggcgagaaagatctgagcaaattaaccagccagatctacatctacgccatcccgtacctgtgggcctttcctccggaagagcagatcttcggtacaagtgccattgtgccgcgtcatgttcgtcgcgcaggccgtaataccgttgatcctaccgttaagaactaccagtggggtgatctgaccgcagcttcttttgaagcaaaagatcgtggcgcccgcaccgcaatcctgctggatgcagacaactgtgtggccgagggtccgggctttaacgtggtgatggtgaaggatggcaaactgagtagcccgagccgtaatgccctgccgggtattacacgtctgaccgtgatggagatggccgatgaaatgggcatcgaattcaccctgcgcgatatcaccagccgtgagttatatgaggccgacgaactgatcgccgtgaccaccgcaggtggcattaccccgattaccagtctggatggcgaaccgctgggcgatggtacccctggtcctgtgacagtggccattcgcgatcgcttttgggccatgatggatgagccgagcagtctggtggaggccattgaatattaa

SEQ ID NO: 45 - DNA, 1026 bp, (Actinobacteria sp.)
atgaccattagcaaagacattgactatagcaccagcaacctggtgagtgtggccccgggtgcaatccgtgaacctaccccggcaggcagcgtgatccagtacagtgactacgagctggatgaaagcagcccgtttgccggtggtgcagcctggattgaaggtgagtatgttccggcagcagaggcccgtattagcctgtttgataccggcttcggccatagcgatctgacctacaccgttgcccatgtttggcacggcaacatctttcgcctgaaagaccacattgaccgcgtgtttgatggcgcccagaaactgcgtatacagagcccgctgaccaaggccgaagtggaggatattaccaaacgctgcgtgagcctgagtcagctgcgcgagagcttcgtgaacatcaccattacccgcggttatggcgcccgcaaaggcgagaaagatctgagcaaattaaccagccagatctacatctacgccatcccgtacctgtgggcctttcctccggaagagcagatcttcggtacaagtgccattgtgccgcgtcatgttcgtcgcgcaggccgtaataccgttgatcctaccgttaagaactaccagtggggtgatctgaccgcagcttcttttgaagcaaaagatcgtggcgcccgcaccgcaatcctgctggatgcagacaactgtgtggccgagggtccgggctttaacgtggtgatggtgaaggatggcaaactgagtagcccgagccgtaatgccctgccgggtattacacgtctgaccgtgatggagatggccgatgaaatgggcatcgaattcaccctgcgcgatatcaccagccgtgagttatatgaggccgacgaactgatcgccgtgaccaccgcaggtggcattaccccgattaccagtctggatggcgaaccgctgggcgatggtacccctggtcctgtgacagtggccattcgcgatcgcttttgggccatgatggatgagccgagcagtctggtggaggccattgaatattaa

SEQ ID NO: 46 - DNA, 1026 bp, (Actinobacteria sp.)
atgaccattagcaaagacattgactatagcaccagcaacctggtgagtgtggccccgggtgcaatccgtgaacctaccccggcaggcagcgtgatccagtacagtgactacgagctggatgaaagcagcccgtttgccggtggtgcagcctggattgaaggtgagtatgttccggcagcagaggcccgtattagcctgtttgataccggcttcggccatagcgatctgacctacaccgttgcccatgtttggcacggcaacatctttcgcctgggagaccacattgaccgcgtgtttgatggcgcccagaaactgcgtctgcagagcccgctgaccaaggccgaagtggaggatattaccaaacgctgcgtgagcctgagtcagctgcgcgagagcttcgtgaacatcaccattacccgcggttatggcgcccgcaaaggcgagaaagatctgagcaaattaaccagccagatctacatctacgccatcccgtacctgtgggcctttcctccggaagagcagatcttcggtacaagtgccattgtgccgcgtcatgttcgtcgcgcaggccgtaataccgttgatcctaccgttaagaactaccagtggggtgatctgaccgcagcttcttttgaagcaaaagatcgtggcgcccgcaccgcaatcctgctggatgcagacaactgtgtggccgagggtccgggctttaacgtggtgatggtgaaggatggcaaactgagtagcccgagccgtaatgccctgccgggtattacacgtctgaccgtgatggagatggccgatgaaatgggcatcgaattcaccctgcgcgatatcaccagccgtgagttatatgaggccgacgaactgatcgccgtgaccaccgcaggtggcattaccccgattaccagtctggatggcgaaccgctgggcgatggtacccctggtcctgtgacagtggccattcgcgatcgcttttgggccatgatggatgagccgagcagtctggtggaggccattgaatattaa

SEQ ID NO: 47 - DNA, 1026 bp, (Actinobacteria sp.)
atgaccattagcaaagacattgactatagcaccagcaacctggtgagtgtggccccgggtgcaatccgtgaacctaccccggcaggcagcgtgatccagtacagtgactacgagctggatgaaagcagcccgtttgccggtggtgcagcctggattgaaggtgagtatgttccggcagcagaggcccgtattagcctgtttgataccggcttcggccatagcgatctgacctacaccgttgcccatgtttggcacggcaacatctttcgcctgaaagaccacattgaccgcgtgtttgatggcgcccagaaactgcgtctgcagagcccgctgaccaaggccgaagtggaggatattaccaaacgctgcgtggccctgagtcagctgcgcgagagcttcgtgaacatcaccattacccgcggttatggcgcccgcaaaggcgagaaagatctgagcaaattaaccagccagatctacatctacgccatcccgtacctgtgggcctttcctccggaagagcagatcttcggtacaagtgccattgtgccgcgtcatgttcgtcgcgcaggccgtaataccgttgatcctaccgttaagaactaccagtggggtgatctgaccgcagcttcttttgaagcaaaagatcgtggcgcccgcaccgcaatcctgctggatgcagacaactgtgtggccgagggtccgggctttaacgtggtgatggtgaaggatggcaaactgagtagcccgagccgtaatgccctgccgggtattacacgtctgaccgtgatggagatggccgatgaaatgggcatcgaattcaccctgcgcgatatcaccagccgtgagttatatgaggccgacgaactgatcgccgtgaccaccgcaggtggcattaccccgattaccagtctggatggcgaaccgctgggcgatggtacccctggtcctgtgacagtggccattcgcgatcgcttttgggccatgatggatgagccgagcagtctggtggaggccattgaatattaa

SEQ ID NO: 48 - DNA, 1026 bp, (Actinobacteria sp.)
atgaccattagcaaagacattgactatagcaccagcaacctggtgagtgtggccccgggtgcaatccgtgaacctaccccggcaggcagcgtgatccagtacagtgactacgagctggatgaaagcagcccgtttgccggtggtgcagcctggattgaaggtgagtatgttccggcagcagaggcccgtattagcctgtttgataccggcttcggccatagcgatctgacctacaccgttgcccatgtttggcacggcaacatctttcgcctgaaagaccacattgaccgcgtgtttgatggcgcccagaaactgcgtctgcagagcccgctgaccaaggccgaagtggaggatattaccaaacgctgcgtgagcctgagtcagctgcgcgaggccttcgtgaacatcaccattacccgcggttatggcgcccgcaaaggcgagaaagatctgagcaaattaaccagccagatctacatctacgccatcccgtacctgtgggcctttcctccggaagagcagatcttcggtacaagtgccattgtgccgcgtcatgttcgtcgcgcaggccgtaataccgttgatcctaccgttaagaactaccagtggggtgatctgaccgcagcttcttttgaagcaaaagatcgtggcgcccgcaccgcaatcctgctggatgcagacaactgtgtggccgagggtccgggctttaacgtggtgatggtgaaggatggcaaactgagtagcccgagccgtaatgccctgccgggtattacacgtctgaccgtgatggagatggccgatgaaatgggcatcgaattcaccctgcgcgatatcaccagccgtgagttatatgaggccgacgaactgatcgccgtgaccaccgcaggtggcattaccccgattaccagtctggatggcgaaccgctgggcgatggtacccctggtcctgtgacagtggccattcgcgatcgcttttgggccatgatggatgagccgagcagtctggtggaggccattgaatattaa

SEQ ID NO: 49 - DNA, 1026 bp, (Actinobacteria sp.)
atgaccattagcaaagacattgactatagcaccagcaacctggtgagtgtggccccgggtgcaatccgtgaacctaccccggcaggcagcgtgatccagtacagtgactacgagctggatgaaagcagcccgtttgccggtggtgcagcctggattgaaggtgagtatgttccggcagcagaggcccgtattagcctgtttgataccggcttcggccatagcgatctgacctacaccgttgcccatgtttggcacggcaacatctttcgcctgaaagaccacattgaccgcgtgtttgatggcgcccagaaactgcgtctgcagagcccgctgaccaaggccgaagtggaggatattaccaaacgctgcgtgagcctgagtcagctgcgcgagagcttcgtgaacatcaccattacccgcggttatggcgcccgcaaaggcgagaaagatctgagcaaattaaccagccagatctacatctacgccatcccgtacctgtgggcctttcctccggaagagcagatcttcggtacaagtgccattgtgccgcgtcatgttcgtcgcgcaggccgtaataccgttgatcctaccgttaagaactaccagtggggtgatctgaccgcagcttcttttgaagcaaaagatcgtggcgcccgcaccgcaatcctgctggatggagacaactgtgtggccgagggtccgggctttaacgtggtgatggtgaaggatggcaaactgagtagcccgagccgtaatgccctgccgggtattacacgtctgaccgtgatggagatggccgatgaaatgggcatcgaattcaccctgcgcgatatcaccagccgtgagttatatgaggccgacgaactgatcgccgtgaccaccgcaggtggcattaccccgattaccagtctggatggcgaaccgctgggcgatggtacccctggtcctgtgacagtggccattcgcgatcgcttttgggccatgatggatgagccgagcagtctggtggaggccattgaatattaa

SEQ ID NO: 50 - DNA, 1026 bp, (Actinobacteria sp.)
atgaccattagcaaagacattgactatagcaccagcaacctggtgagtgtggccccgggtgcaatccgtgaacctaccccggcaggcagcgtgatccagtacagtgactacgagctggatgaaagcagcccgtttgccggtggtgcagcctggattgaaggtgagtatgttccggcagcagaggcccgtattagcctgtttgataccggcttcggccatagcgatctgacctacaccgttgcccatgtttggcacggcaacatctttcgcctgaaagaccacattgaccgcgtgtttgatggcgcccagaaactgcgtctgcagagcccgctgaccaaggccgaagtggaggatattaccaaacgctgcgtgagcctgagtcagctgcgcgagagcttcgtgaacatcaccattacccgcggttatggcgcccgcaaaggcgagaaagatctgagcaaattaaccagccagatctacatctacgccatcccgtacctgtgggcctttcctccggaagagcagatcttcggtacaagtgccattgtgccgcgtcatgttcgtcgcgcaggccgtaataccgttgatcctaccgttaagaactaccagtggggtgatctgaccgcagcttcttttgaagcaaaagatcgtggcgcccgcaccgcaatcctgctggatgcagacaactgtgtggccgagggtccgggctttaacgtggtgatggtgaaggatggcaaactgagtagcccgagccgtaatgccctgccgggtattacacgtctgaccgtgatggagatggccgatgaaatgggcatcgaattcaccctgcgcgatatcaccagccgtgagttatatgaggccgacgaactgatcgcctgcaccaccgcaggtggcattaccccgattaccagtctggatggcgaaccgctgggcgatggtacccctggtcctgtgacagtggccattcgcgatcgcttttgggccatgatggatgagccgagcagtctggtggaggccattgaatattaa

SEQ ID NO: 51 - DNA, 1026 bp, (Actinobacteria sp.)
atgaccattagcaaagacattgactatagcaccagcaacctggtgagtgtggccccgggtgcaatccgtgaacctaccccggcaggcagcgtgatccagtacagtgactacgagctggatgaaagcagcccgtttgccggtggtgcagcctggattgaaggtgagtatgttccggcagcagaggcccgtattagcctgtttgataccggcttcggccatagcgatctgacctacaccgttgcccatgtttggcacggcaacatctttcgcctgaaagaccacattgaccgcgtgtttgatggcgcccagaaactgcgtctgcagagcccgctgaccaaggccgaagtggaggatattaccaaacgctgcgtgagcctgagtcagctgcgcgagagcttcgtgaacatcaccattacccgcggttatggcgcccgcaaaggcgagaaagatctgagcaaattaaccagccagatctacatctacgccatcccgtacctgtgggcctttcctccggaagagcagatcttcggtacaagtgccattgtgccgcgtcatgttcgtcgcgcaggccgtaataccgttgatcctaccgttaagaactaccagtggggtgatctgaccgcagcttcttttgaagcaaaagatcgtggcgcccgcaccgcaatcctgctggatgcagacaactgtgtggccgagggtccgggctttaacgtggtgatggtgaaggatggcaaactgagtagcccgagccgtaatgccctgccgggtattacacgtctgaccgtgatggagatggccgatgaaatgggcatcgaattcaccctgcgcgatatcaccagccgtgagttatatgaggccgacgaactgatcgccgtgaccaccggaggtggcattaccccgattaccagtctggatggcgaaccgctgggcgatggtacccctggtcctgtgacagtggccattcgcgatcgcttttgggccatgatggatgagccgagcagtctggtggaggccattgaatattaa

SEQ ID NO: 52 - DNA, 1026 bp, (Actinobacteria sp.)
atgaccattagcaaagacattgactatagcaccagcaacctggtgagtgtggcctcgggtgcaatccgtgaacctaccccggcaggcagcgtgatccagtacagtgactacgagctggatgaaagcagcccgtttgccggtggtgcagcctggattgaaggtgagtatgttccggcagcagaggcccgtattagcctgtttgataccggcttcggccatagcgatctgacctacaccgttgcccatgtttggcacggcaacatctttcgcctgaaagaccacattgaccgcgtgtttgatggcgcccagaaactgcgtctgcagagcccgctgaccaaggccgaagtggaggatattaccaaacgctgcgtgagcctgagtcagctgcgcgagagcttcgtgaacatcaccattacccgcggttatggcgcccgcaaaggcgagaaagatctgagcaaattaaccagccagatctacatctacgccatcccgtacctgtgggcctttcctccggaagagcagatcttcggtacaagtgccattgtgccgcgtcatgttcgtcgcgcaggccgtaataccgttgatcctaccgttaagaactaccagtggggtgatctgaccgcagcttcttttgaagcaaaagatcgtggcgcccgcaccgcaatcctgctggatgcagacaactgtgtggccgagggtccgggctttaacgtggtgatggtgaaggatggcaaactgagtagcccgagccgtaatgccctgccgggtattacacgtctgaccgtgatggagatggccgatgaaatgggcatcgaattcaccctgcgcgatatcaccagccgtgagttatatgaggccgacgaactgatcgccgtgaccaccgcaggtggcattaccccgattaccagtctggatggcgaaccgctgggcgatggtacccctggtcctgtgacagtggccattcgcgatcgcttttgggccatgatggatgagccgagcagtctggtggaggccattgaatattaa

SEQ ID NO: 53 - DNA, 1026 bp, (Actinobacteria sp.)
atgaccattagcaaagacattgactatagcaccagcaacctggtgagtgtggccccgggtgcaatccgtgaacctaccccggcaggcagcgtgatccagtacagtgactacgagctggattcaagcagcccgtttgccggtggtgcagcctggattgaaggtgagtatgttccggcagcagaggcccgtattagcctgtttgataccggcttcggccatagcgatctgacctacaccgttgcccatgtttggcacggcaacatctttcgcctgaaagaccacattgaccgcgtgtttgatggcgcccagaaactgcgtctgcagagcccgctgaccaaggccgaagtggaggatattaccaaacgctgcgtgagcctgagtcagctgcgcgagagcttcgtgaacatcaccattacccgcggttatggcgcccgcaaaggcgagaaagatctgagcaaattaaccagccagatctacatctacgccatcccgtacctgtgggcctttcctccggaagagcagatcttcggtacaagtgccattgtgccgcgtcatgttcgtcgcgcaggccgtaataccgttgatcctaccgttaagaactaccagtggggtgatctgaccgcagcttcttttgaagcaaaagatcgtggcgcccgcaccgcaatcctgctggatgcagacaactgtgtggccgagggtccgggctttaacgtggtgatggtgaaggatggcaaactgagtagcccgagccgtaatgccctgccgggtattacacgtctgaccgtgatggagatggccgatgaaatgggcatcgaattcaccctgcgcgatatcaccagccgtgagttatatgaggccgacgaactgatcgccgtgaccaccgcaggtggcattaccccgattaccagtctggatggcgaaccgctgggcgatggtacccctggtcctgtgacagtggccattcgcgatcgcttttgggccatgatggatgagccgagcagtctggtggaggccattgaatattaa

SEQ ID NO: 54 - DNA, 1026 bp, (Actinobacteria sp.)
atgaccattagcaaagacattgactatagcaccagcaacctggtgagtgtggccccgggtgcaatccgtgaacctaccccggcaggcagcgtgatccagtacagtgactacgagctggatgaaagcaacccgtttgccggtggtgcagcctggattgaaggtgagtatgttccggcagcagaggcccgtattagcctgtttgataccggcttcggccatagcgatctgacctacaccgttgcccatgtttggcacggcaacatctttcgcctgaaagaccacattgaccgcgtgtttgatggcgcccagaaactgcgtctgcagagcccgctgaccaaggccgaagtggaggatattaccaaacgctgcgtgagcctgagtcagctgcgcgagagcttcgtgaacatcaccattacccgcggttatggcgcccgcaaaggcgagaaagatctgagcaaattaaccagccagatctacatctacgccatcccgtacctgtgggcctttcctccggaagagcagatcttcggtacaagtgccattgtgccgcgtcatgttcgtcgcgcaggccgtaataccgttgatcctaccgttaagaactaccagtggggtgatctgaccgcagcttcttttgaagcaaaagatcgtggcgcccgcaccgcaatcctgctggatgcagacaactgtgtggccgagggtccgggctttaacgtggtgatggtgaaggatggcaaactgagtagcccgagccgtaatgccctgccgggtattacacgtctgaccgtgatggagatggccgatgaaatgggcatcgaattcaccctgcgcgatatcaccagccgtgagttatatgaggccgacgaactgatcgccgtgaccaccgcaggtggcattaccccgattaccagtctggatggcgaaccgctgggcgatggtacccctggtcctgtgacagtggccattcgcgatcgcttttgggccatgatggatgagccgagcagtctggtggaggccattgaatattaa

SEQ ID NO: 55 - DNA, 935 bp, (Actinobacteria sp.)
tgatccagtacagtgactacgagctggatgaaagcagcccgtttgccggtggtgcagcctggattgaaggtgagtatgttccggcagcagaggcccgtattagcctgtttgataccggcttcggccatagcgatctgacctacaccgttgcccatgtttggcacggcaacatctttcgcctgaaagaccacattgaccgcgtgtttgatggcgcccagaaactgcgtctgcagagcccgctgaccaaggccgaagtggaggatattaccaaacgctgcgtgagcctgagtcagctgcgcgagagcttcgtgaacatcaccattacccgcggttatggcgcccgcaaaggcgagaaagatctgagcaaattaaccagccagatctacatctacgccatcccgtacctgtgggcctttcctccggaagagcagatcttcggtacaagtgccattgtgccgcgtcatgttcgtcgcgcaggccgtaataccgttgatcctaccgttaagaactaccagtggggtgatctgaccgcagcttcttttgaagcaaaagatcgtggcgcccgcaccgcaatcctgctggatgcagacaactgtgtggccgagggtccgggctttaacgtggtgatggtgaaggatggcaaactgagtagcccgagccgtaatgccctgccgggtattacacgtctgaccgtgatggagatggccgatgaaatgggcatcgaattcaccctgcgcgatatcaccagccgtgagttatatgaggccgacgaactgatcgccgtgaccaccgcaggtggcattaccccgattaccagtctggatggcgaatcgctgggcgatggtacccctggtcctgtgacagtggccattcgcgatcgcttttgggccatgatggatgagccgagcagtctggtggaggccattgaatattaa

SEQ ID NO: 56 - DNA, 1026 bp, (Actinobacteria sp.)
atgaccattagcaaagacattgactatagcaccagcaacctggtgagtgtggccccgggtgcaatccgtgaacctaccccggcaggcagcgtgatccagtacagtgactacgagctggatgaaagcagcccgtttgccggtggtgcagcctggattgaaggtgagtatgttccggcagcagaggcccgtattagcctgtttgataccggcttcggccatagcgatctgacctacaccgttgcccatgtttggcacggcaacatctttcgcctgaaagaccacattgaccgcgtgtttgatggcgcccagaaactgcgtctgcagagcccgctgaccaaggccgaagtggaggatattaccaaacgctgcgtgagcctgagtcagctgcgcgagagcttcgtgaacatcaccattacccgcggttatggcgcccgcaaaggcgagaaagatctgagcaaattaaccagccagatctacatctacgccatcccgtacctgtgggcctttcctccggaagagcagatcttcggtacaagtgccattgtgccgcgtcatgttcgtcgcgcaggccgtaataccgttgatcctaccgttaagaactaccagtggggtgatctgaccgcagcttcttttgaagcaaaagatcgtggcgcccgcaccgcaatcctgctggatgcagacaactgtgtggccgagggtccgggctttaacgtggtgatggtgaaggatggcaaactgagtagcccgagccgtaatgccctgccgggtattacacgtctgaccgtgatggagatggccgatgaaatgggcatcgaattcaccctgcgcgatatcaccagccgtgagttatatgaggccgacgaactgatcgccgtgaccaccgcaggtggcattaccccgattaccagtctggatggcgaaccgctgggcgatggtacccctggtcctgtgacagtggccattcgcgatcgcttttgggccatgatggatgagtcgagcagtctggtggaggccattgaatattaa

SEQ ID NO: 57 - DNA, 1026 bp, (Actinobacteria sp.)
atgaccattagcaaagacattgactatagcaccagcaacctggtgagtgtggccccgggtgcaatccgtgaacctaccccggcaggcagcgtgatccagtacagtgactacgagctggatgaaagcagcccgtttgccggtggtgcagcctggattgaaggtgagtatgttccggcagcagaggcccgtattagcctgtttgataccggcttcggccatagcgatgcgacctacaccgttgcccatgtttggcacggcaacatctttcgcctgaaagaccacattgaccgcgtgtttgatggcgcccagaaactgcgtatacagagccagctgaccaaggccgaagtggaggatattaccaaacgctgcgtgagcctgagtcagctgcgcgagagcttcgtgaacatcaccattacccgcggttatggcgcccgcaaaggcgagaaagatctgagcaaattaaccagccagatctacatctacgccatcccgtacctgtgggcctttcctccggaagagcagatcttcggtacaagtgccattgtgccgcgtcatgttcgtcgcgcaggccgtaataccgttgatcctaccgttaagaactaccagtggggtgatctgaccgcagcttcttttgaagcaaaagatcgtggcgcccgcaccgcaatcctgctggatgcagacaactgtgtggccgagggtccgggctttaacgtggtgatggtgaaggatggcaaactgagtagcccgagccgtaatgccctgccgggtattacacgtctgaccgtgatggagatggccgatgaaatgggcatcgaattcaccctgcgcgatatcaccagccgtgagttatatgaggccgacgaactgatcgccgtgaccaccgcaggtggcattaccccgattaccagtctggatggcgaaccgctgggcgatggtacccctggtcctgtgacagtggccattcgcgatcgcttttgggccatgatggatgagccgagcagtctggtggaggccattgaatattaa

SEQ ID NO: 58 - DNA, 1026 bp, (Actinobacteria sp.)
atgaccattagcaaagacattgactatagcaccagcaacctggtgagtgtggccccgggtgcaatccgtgaacctaccccggcaggcagcgtgatccagtacagtgactacgagctggatgaaagcagcccgtttgccggtggtgcagcctggattgaaggtgagtatgttccggcagcagaggcccgtattagcctgtttgataccggcttcggccatagcgatgcgacctacaccgttgcccatgtttggcacggcaacatctttcgcctgaaagaccacattgaccgcgtgtttgatggcgcccagaaactgcgtctgcagagcccgctgaccaaggccgaagtggaggatattaccaaacgctgcgtggccctgagtcagctgcgcgagagcttcgtgaacatcaccattacccgcggttatggcgcccgcaaaggcgagaaagatctgagcaaattaaccagccagatctacatctacgccatcccgtacctgtgggcctttcctccggaagagcagatcttcggtacaagtgccattgtgccgcgtcatgttcgtcgcgcaggccgtaataccgttgatcctaccgttaagaactaccagtggggtgatctgaccgcagcttcttttgaagcaaaagatcgtggcgcccgcaccgcaatcctgctggatggagacaactgtgtggccgagggtccgggctttaacgtggtgatggtgaaggatggcaaactgagtagcccgagccgtaatgccctgccgggtattacacgtctgaccgtgatggagatggccgatgaaatgggcatcgaattcaccctgcgcgatatcaccagccgtgagttatatgaggccgacgaactgatcgccgtgaccaccgcaggtggcattaccccgattaccagtctggatggcgaaccgctgggcgatggtacccctggtcctgtgacagtggccattcgcgatcgcttttgggccatgatggatgagccgagcagtctggtggaggccattgaatattaa

SEQ ID NO: 59 - DNA, 1026 bp, (Actinobacteria sp.)
atgaccattagcaaagacattgactatagcaccagcaacctggtgagtgtggccccgggtgcaatccgtgaacctaccccggcaggcagcgtgatccagtacagtgactacgagctggatgaaagcagcccgtttgccggtggtgcagcctggattgaaggtgagtatgttccggcagcagaggcccgtattagcctgtttgataccggcttcggccatagcgatgcgacctacagcgttgcccatgtttggcacggcaacatctttcgcctgaaagaccacattgaccgcgtgtttgatggcgcccagaaactgcgtctgcagagcccgctgaccaaggccgaagtggaggatattaccaaacgctgcgtgagcctgagtcagctgcgcgagagcttcgtgaacatcaccattacccgcggttatggcgcccgcaaaggcgagaaagatctgagcaaattaaccagccagatctacatctacgccatcccgtacctgtgggcctttcctccggaagagcagatcttcggtacaagtgccattgtgccgcgtcatgttcgtcgcgcaggccgtaataccgttgatcctaccgttaagaactaccagtggggtgatctgaccgcagcttcttttgaagcaaaagatcgtggcgcccgcaccgcaatcctgctggatgcagacaactgtgtggccgagggtccgggctttaacgtggtgatggtgaaggatggcaaactgagtagcccgagccgtaatgccctgccgggtattacacgtctgaccgtgatggagatggccgatgaaatgggcatcgaattcaccctgcgcgatatcaccagccgtgagttatatgaggccgacgaactgatcgccgtgaccaccggaggtggcattaccccgattaccagtctggatggcgaaccgctgggcgatggtacccctggtcctgtgacagtggccattcgcgatcgcttttgggccatgatggatgagccgagcagtctggtggaggccattgaatattaa

SEQ ID NO: 60 - DNA, 1026 bp, (Actinobacteria sp.)
atgaccattagcaaagacattgactatagcaccagcaacctggtgagtgtggccccgggtgcaatccgtgaacctaccccggcaggcagcgtgatccagtacagtgactacgagctggatgaaagcagcccgtttgccggtggtgcagcctggattgaaggtgagtatgttccggcagcagaggcccgtattagcctgtttgataccggcttcggccatagcgatgcgacctacaccgttgcccatgtttggcacggcaacatctttcgcctgaaagaccacattgaccgcgtgtttgatggcgcccagaaactgcgtatacagagccagctgaccaaggccgaagtggaggatattaccaaacgctgcgtgagcctgagtcagctgcgcgagagcttcgtgaacatcaccattacccgcggttatggcgcccgcaaaggcgagaaaggtctgagcaaattaaccagccagatctacatctacgccatcccgtacctgtgggcctttcctccggaagagcagatcttcggtacaagtgccattgtgccgcgtcatgttcgtcgcgcaggccgtaataccgttgatcctaccgttaagaactaccagtggggtgatctgaccgcagcttcttttgaagcaaaagatcgtggcgcccgcaccgcaatcctgctggatgcagacaactgtgtggccgagggtccgggctttaacgtggtgatggtgaaggatggcaaactgagtagcccgagccgtaatgccctgccgggtattacacgtctgaccgtgatggagatggccgatgaaatgggcatcgaattcaccctgcgcgatatcaccagccgtgagttatatgaggccgacgaactgatcgccgtgaccaccgcaggtggcattaccccgattaccagtctggatggcgaaccgctgggcgatggtacccctggtcctgtgacagtggccattcgcgatcgcttttgggccatgatggatgagccgagcagtctggtggaggccattgaatattaa